European Patent Specification EP 3 684 422 B1, published December 20, 2023. Title: A Gene Therapy Strategy to Restore Electrical and Cardiac Function in Arrhythmic Right Ventricular Cardiomyopathy. Applicant: The Regents of the University of California. The sequence listing filed with the application follows.

SEQUENCE LISTING (12 sequences)

SEQ ID NO: 1 - protein, 382 aa, Homo sapiens
MGDWSALGKLLDKVQAYSTAGGKVWLSVLFIFRILLLGTAVESAWGDEQSAFRCNTQQPGCENVCYDKSFPISHVRFWVLQIIFVSVPTLLYLAHVFYVMRKEEKLNKKEEELKVAQTDGVNVDMHLKQIEIKKFKYGIEEHGKVKMRGGLLRTYIISILFKSIFEVAFLLIQWYIYGFSLSAVYTCKRDPCPHQVDCFLSRPTEKTIFIIFMLVVSLVSLALNIIELFYVFFKGVKDRVKGKSDPYHATSGALSPAKDCGSQKYAYFNGCSSPTAPLSPMSPPGYKLVTGDRNNSSCRNYNKQASEQNWANYSAEQNRMGQAGSTISNSHAQPFDFPDDNQNSKKLAAGHELQPLAIVDQRPSSRASSRASSRPRPDDLEI

SEQ ID NO: 2 - DNA, 1146 bp, Homo sapiens
atgggtgactggagcgccttaggcaaactccttgacaaggttcaagcctactcaactgctggagggaaggtgtggctgtcagtacttttcattttccgaatcctgctgctggggacagcggttgagtcagcctggggagatgagcagtctgcctttcgttgtaacactcagcaacctggttgtgaaaatgtctgctatgacaagtctttcccaatctctcatgtgcgcttctgggtcctgcagatcatatttgtgtctgtacccacactcttgtacctggctcatgtgttctatgtgatgcgaaaggaagagaaactgaacaagaaagaggaagaactcaaggttgcccaaactgatggtgtcaatgtggacatgcacttgaagcagattgagataaagaagttcaagtacggtattgaagagcatggtaaggtgaaaatgcgaggggggttgctgcgaacctacatcatcagtatcctcttcaagtctatctttgaggtggccttcttgctgatccagtggtacatctatggattcagcttgagtgctgtttacacttgcaaaagagatccctgcccacatcaggtggactgtttcctctctcgccccacggagaaaaccatcttcatcatcttcatgctggtggtgtccttggtgtccctggccttgaatatcattgaactcttctatgttttcttcaagggcgttaaggatcgggttaagggaaagagcgacccttaccatgcgaccagtggtgcgctgagccctgccaaagactgtgggtctcaaaaatatgcttatttcaatggctgctcctcaccaaccgctcccctctcgcctatgtctcctcctgggtacaagctggttactggcgacagaaacaattcttcttgccgcaattacaacaagcaagcaagtgagcaaaactgggctaattacagtgcagaacaaaatcgaatggggcaggcgggaagcaccatctctaactcccatgcacagccttttgatttccccgatgataaccagaattctaaaaaactagctgctggacatgaattacagccactagccattgtggaccagcgaccttcaagcagagccagcagtcgtgccagcagcagacctcggcctgatgacctggagatc

SEQ ID NO: 3 - protein, 281 aa, Homo sapiens
MRKEEKLNKKEEELKVAQTDGVNVDMHLKQIEIKKFKYGIEEHGKVKMRGGLLRTYIISILFKSIFEVAFLLIQWYIYGFSLSAVYTCKRDPCPHQVDCFLSRPTEKTIFIIFMLVVSLVSLALNIIELFYVFFKGVKDRVKGKSDPYHATSGALSPAKDCGSQKYAYFNGCSSPTAPLSPMSPPGYKLVTGDRNNSSCRNYNKQASEQNWANYSAEQNRMGQAGSTISNSHAQPFDFPDDNQNSKKLAAGHELQPLAIVDQRPSSRASSRASSRPRPDDL

SEQ ID NO: 4 - protein, 258 aa, Homo sapiens [sequence omitted]

SEQ ID NO: 5 - protein, 236 aa, Homo sapiens
MRGGLLRTYIISILFKSIFEVAFLLIQWYIYGFSLSAVYTCKRDPCPHQVDCFLSRPTEKTIFIIFMLVVSLVSLALNIIELFYVFFKGVKDRVKGKSDPYHATSGALSPAKDCGSQKYAYFNGCSSPTAPLSPMSPPGYKLVTGDRNNSSCRNYNKQASEQNWANYSAEQNRMGQAGSTISNSHAQPFDFPDDNQNSKKLAAGHELQPLAIVDQRPSSRASSRASSRPRPDDLEI

SEQ ID NO: 6 - protein, 170 aa, Homo sapiens [sequence omitted]

SEQ ID NO: 7 - DNA, 9215 bp, Artificial Sequence
  Adeno cx43 vector
catcatcaataatataccttattttggattgaagccaatatgataatgagggggtggagtttgtgacgtggcgcggggcgtgggaacggggcgggtgacgtagtagtgtggcggaagtgtgatgttgcaagtgtggcggaacacatgtaagcgacggatgtggcaaaagtgacgtttttggtgtgcgccggtgtacacaggaagtgacaattttcgcgcggttttaggcggatgttgtagtaaatttgggcgtaaccgagtaagatttggccattttcgcgggaaaactgaataagaggaagtgaaatctgaataattttgtgttactcatagcgcgtaatactgtaatagtaatcaattacggggtcattagttcatagcccatatatggagttccgcgttacataacttacggtaaatggcccgcctggctgaccgcccaacgacccccgcccattgacgtcaataatgacgtatgttcccatagtaacgccaatagggactttccattgacgtcaatgggtggagtatttacggtaaactgcccacttggcagtacatcaagtgtatcatatgccaagtacgccccctattgacgtcaatgacggtaaatggcccgcctggcattatgcccagtacatgaccttatgggactttcctacttggcagtacatctacgtattagtcatcgctattaccatggtgatgcggttttggcagtacatcaatgggcgtggatagcggtttgactcacggggatttccaagtctccaccccattgacgtcaatgggagtttgttttggcaccaaaatcaacgggactttccaaaatgtcgtaacaactccgccccattgacgcaaatgggcggtaggcgtgtacggtgggaggtctatataagcagagctggtttagtgaaccgtcagatccgctagattaagtaatacgactcactataggcatggatgggtgactggagcgccttaggcaaactccttgacaaggttcaagcctactcaactgctggagggaaggtgtggctgtcagtacttttcattttccgaatcctgctgctggggacagcggttgagtcagcctggggagatgagcagtctgcctttcgttgtaacactcagcaacctggttgtgaaaatgtctgctatgacaagtctttcccaatctctcatgtgcgcttctgggtcctgcagatcatatttgtgtctgtacccacactcttgtacctggctcatgtgttctatgtgatgcgaaaggaagagaaactgaacaagaaagaggaagaactcaaggttgcccaaactgatggtgtcaatgtggacatgcacttgaagcagattgagataaagaagttcaagtacggtattgaagagcatggtaaggtgaaaatgcgaggggggttgctgcgaacctacatcatcagtatcctcttcaagtctatctttgaggtggccttcttgctgatccagtggtacatctatggattcagcttgagtgctgtttacacttgcaaaagagatccctgcccacatcaggtggactgtttcctctctcgccccacggagaaaaccatcttcatcatcttcatgctggtggtgtccttggtgtccctggccttgaatatcattgaactcttctatgttttcttcaagggcgttaaggatcgggttaagggaaagagcgacccttaccatgcgaccagtggtgcgctgagccctgccaaagactgtgggtctcaaaaatatgcttatttcaatggctgctcctcaccaaccgctcccctctcgcctatgtctcctcctgggtacaagctggttactggcgacagaaacaattcttcttgccgcaattacaacaagcaagcaagtgagcaaaactgggctaattacagtgcagaacaaaatcgaatggggcaggcgggaagcaccatctctaactcccatgcacagccttttgatttccccgatgatctagccaattcccgtgtgagcaagggcgaggagctgttcaccggggtggtgcccatcctggtcgagctggacggcgacgtaaacggccacaagttcagcgtgtccggcgagggcgagggcgatgccacctacggcaagctgaccctgaagttcatctgcaccaccggcaagctgcccgtgccctggcccaccctcgtgaccaccttcggctacggcgtgcagtgcttcgcccgctaccccgaccacatgcgccagcacgacttcttcaagtccgccatgcccgaaggctacgtccaggagcgcaccatcttcttcaaggacgacggcaactacaagacccgcgccgaggtgaagttcgagggcgacaccctggtgaaccgcatcgagctgaagggcatcgacttcaaggaggacggcaacatcctggggcacaagctggagtacaactacaacagccacaacgtctatatcatggccgacaagcagaagaacggcatcaaggtgaacttcaagatccgccacaacatcgaggacggcagcgtgcagctcgccgaccactaccagcagaacacccccatcggcgacggccccgtgctgctgcccgacaaccactacctgagctaccagtccgccctgagcaaagaccccaacgagaagcgcgatcacatggtcctgctggagttcgtgaccgccgccgggatcactctcggcatggacgagctgtacaagtaagcttctagataagatatccgatccaccggatctagataactgatcataatcagccataccacatttgtagaggttttacttgctttaaaaaacctcccacacctccccctgaacctgaaacataaaatgaatgcaattgttgttgttaacttgtttattgcagcttataatggttacaaataaagcaatagcatcacaaatttcacaaataaagcatttttttcactgcattctagttgtggtttgtccaaactcatcaatgtatcttaacgcggatctgggcgtggttaagggtgggaaagaatatataaggtgggggtcttatgtagttttgtatctgttttgcagcagccgccgccgccatgagcaccaactcgtttgatggaagcattgtgagctcatatttgacaacgcgcatgcccccatgggccggggtgcgtcagaatgtgatgggctccagcattgatggtcgccccgtcctgcccgcaaactctactaccttgacctacgagaccgtgtctggaacgccgttggagactgcagcctccgccgccgcttcagccgctgcagccaccgcccgcgggattgtgactgactttgctttcctgagcccgcttgcaagcagtgcagcttcccgttcatccgcccgcgatgacaagttgacggctcttttggcacaattggattctttgacccgggaacttaatgtcgtttctcagcagctgttggatctgcgccagcaggtttctgccctgaaggcttcctcccctcccaatgcggtttaaaacataaataaaaaaccagactctgtttggatttggatcaagcaagtgtcttgctgtctttatttaggggttttgcgcgcgcggtaggcccgggaccagcggtctcggtcgttgagggtcctgtgtattttttccaggacgtggtaaaggtgactctggatgttcagatacatgggcataagcccgtctctggggtggaggtagcaccactgcagagcttcatgctgcggggtggtgttgtagatgatccagtcgtagcaggagcgctgggcgtggtgcctaaaaatgtctttcagtagcaagctgattgccaggggcaggcccttggtgtaagtgtttacaaagcggttaagctgggatgggtgcatacgtggggatatgagatgcatcttggactgtatttttaggttggctatgttcccagccatatccctccggggattcatgttgtgcagaaccaccagcacagtgtatccggtgcacttgggaaatttgtcatgtagcttagaaggaaatgcgtggaagaacttggagacgcccttgtgacctccaagattttccatgcattcgtccataatgatggcaatgggcccacgggcggcggcctgggcgaagatatttctgggatcactaacgtcatagttgtgttccaggatgagatcgtcataggccatttttacaaagcgcgggcggagggtgccagactgcggtataatggttccatccggcccaggggcgtagttaccctcacagatttgcatttcccacgctttgagttcagatggggggatcatgtctacctgcggggcgatgaagaaaacggtttccggggtaggggagatcagctgggaagaaagcaggttcctgagcagctgcgacttaccgcagccggtgggcccgtaaatcacacctattaccggctgcaactggtagttaagagagctgcagctgccgtcatccctgagcaggggggccacttcgttaagcatgtccctgactcgcatgttttccctgaccaaatccgccagaaggcgctcgccgcccagcgatagcagttcttgcaaggaagcaaagtttttcaacggtttgagaccgtccgccgtaggcatgcttttgagcgtttgaccaagcagttccaggcggtcccacagctcggtcacctgctctacggcatctcgatccagcatatctcctcgtttcgcgggttggggcggctttcgctgtacggcagtagtcggtgctcgtccagacgggccagggtcatgtctttccacgggcgcagggtcctcgtcagcgtagtctgggtcacggtgaaggggtgcgctccgggctgcgcgctggccagggtgcgcttgaggctggtcctgctggtgctgaagcgctgccggtcttcgccctgcgcgtcggccaggtagcatttgaccatggtgtcatagtccagcccctccgcggcgtggcccttggcgcgcagcttgcccttggaggaggcgccgcacgaggggcagtgcagacttttgagggcgtagagcttgggcgcgagaaataccgattccggggagtaggcatccgcgccgcaggccccgcagacggtctcgcattccacgagccaggtgagctctggccgttcggggtcaaaaaccaggtttcccccatgctttttgatgcgtttcttacctctggtttccatgagccggtgtccacgctcggtgacgaaaaggctgtccgtgtccccgtatacagacttgagagggagtttaaacgaattcaatagcttgttgcatgggcggcgatataaaatgcaaggtgctgctcaaaaaatcaggcaaagcctcgcgcaaaaaagaaagcacatcgtagtcatgctcatgcagataaaggcaggtaagctccggaaccaccacagaaaaagacaccatttttctctcaaacatgtctgcgggtttctgcataaacacaaaataaaataacaaaaaaacatttaaacattagaagcctgtcttacaacaggaaaaacaacccttataagcataagacggactacggccatgccggcgtgaccgtaaaaaaactggtcaccgtgattaaaaagcaccaccgacagctcctcggtcatgtccggagtcataatgtaagactcggtaaacacatcaggttgattcacatcggtcagtgctaaaaagcgaccgaaatagcccgggggaatacatacccgcaggcgtagagacaacattacagcccccataggaggtataacaaaattaataggagagaaaaacacataaacacctgaaaaaccctcctgcctaggcaaaatagcaccctcccgctccagaacaacatacagcgcttccacagcggcagccataacagtcagccttaccagtaaaaaagaaaacctattaaaaaaacaccactcgacacggcaccagctcaatcagtcacagtgtaaaaaagggccaagtgcagagcgagtatatataggactaaaaaatgacgtaacggttaaagtccacaaaaaacacccagaaaaccgcacgcgaacctacgcccagaaacgaaagccaaaaaacccacaacttcctcaaatcgtcacttccgttttcccacgttacgtcacttcccattttaagaaaactacaattcccaacacatacaagttactccgccctaaaacctacgtcacccgccccgttcccacgccccgcgccacgtcacaaactccaccccctcattatcatattggcttcaatccaaaataaggtatattattgatgatgttaattaacatgcatggatccatatgcggtgtgaaataccgcacagatgcgtaaggagaaaataccgcatcaggcgctcttccgcttcctcgctcactgactcgctgcgctcggtcgttcggctgcggcgagcggtatcagctcactcaaaggcggtaatacggttatccacagaatcaggggataacgcaggaaagaacatgtgagcaaaaggccagcaaaaggccaggaaccgtaaaaaggccgcgttgctggcgtttttccataggctccgcccccctgacgagcatcacaaaaatcgacgctcaagtcagaggtggcgaaacccgacaggactataaagataccaggcgtttccccctggaagctccctcgtgcgctctcctgttccgaccctgccgcttaccggatacctgtccgcctttctcccttcgggaagcgtggcgctttctcatagctcacgctgtaggtatctcagttcggtgtaggtcgttcgctccaagctgggctgtgtgcacgaaccccccgttcagcccgaccgctgcgccttatccggtaactatcgtcttgagtccaacccggtaagacacgacttatcgccactggcagcagccactggtaacaggattagcagagcgaggtatgtaggcggtgctacagagttcttgaagtggtggcctaactacggctacactagaaggacagtatttggtatctgcgctctgctgaagccagttaccttcggaaaaagagttggtagctcttgatccggcaaacaaaccaccgctggtagcggtggtttttttgtttgcaagcagcagattacgcgcagaaaaaaaggatctcaagaagatcctttgatcttttctacggggtctgacgctcagtggaacgaaaactcacgttaagggattttggtcatgagattatcaaaaaggatcttcacctagatccttttaaattaaaaatgaagttttaaatcaatctaaagtatatatgagtaaacttggtctgacagttaccaatgcttaatcagtgaggcacctatctcagcgatctgtctatttcgttcatccatagttgcctgactccccgtcgtgtagataactacgatacgggagggcttaccatctggccccagtgctgcaatgataccgcgagacccacgctcaccggctccagatttatcagcaataaaccagccagccggaagggccgagcgcagaagtggtcctgcaactttatccgcctccatccagtctattaattgttgccgggaagctagagtaagtagttcgccagttaatagtttgcgcaacgttgttgccattgctgcagccatgagattatcaaaaaggatcttcacctagatccttttcacgtagaaagccagtccgcagaaacggtgctgaccccggatgaatgtcagctactgggctatctggacaagggaaaacgcaagcgcaaagagaaagcaggtagcttgcagtgggcttacatggcgatagctagactgggcggttttatggacagcaagcgaaccggaattgccagctggggcgccctctggtaaggttgggaagccctgcaaagtaaactggatggctttcttgccgccaaggatctgatggcgcaggggatcaagctctgatcaagagacaggatgaggatcgtttcgcatgattgaacaagatggattgcacgcaggttctccggccgcttgggtggagaggctattcggctatgactgggcacaacagacaatcggctgctctgatgccgccgtgttccggctgtcagcgcaggggcgcccggttctttttgtcaagaccgacctgtccggtgccctgaatgaactgcaagacgaggcagcgcggctatcgtggctggccacgacgggcgttccttgcgcagctgtgctcgacgttgtcactgaagcgggaagggactggctgctattgggcgaagtgccggggcaggatctcctgtcatctcaccttgctcctgccgagaaagtatccatcatggctgatgcaatgcggcggctgcatacgcttgatccggctacctgcccattcgaccaccaagcgaaacatcgcatcgagcgagcacgtactcggatggaagccggtcttgtcgatcaggatgatctggacgaagagcatcaggggctcgcgccagccgaactgttcgccaggctcaaggcgagcatgcccgacggcgaggatctcgtcgtgacccatggcgatgcctgcttgccgaatatcatggtggaaaatggccgcttttctggattcatcgactgtggccggctgggtgtggcggaccgctatcaggacatagcgttggctacccgtgatattgctgaagagcttggcggcgaatgggctgaccgcttcctcgtgctttacggtatcgccgctcccgattcgcagcgcatcgccttctatcgccttcttgacgagttcttctgaattttgttaaaatttttgttaaatcagctcattttttaaccaataggccgaaatcggcaccatcccttataaatcaaaagaatagaccgagatagggttgagtgttgttccagtttggaacaagagtccactattaaagaacgtggactccaacgtcaaagggcgaaaaaccgtctatcagggcgatggcccactacgtgaaccatcaccctaatcaagttttttgtggtcgaggtgccgtaaagcactaaatcggaaccctaaagggagcccccgatttagagcttgacggggaaagccggcgaacgtggcgagaaaggaagggaagaaagcgaaaggagcgggcgctagggcgctggcaagtgtagcggtcacgctgcgcgtaaccaccacacccgcgcgcttaatgcgccgctacagggcgcgtccattcgccattcaggatcgaattaattcttaattaa

SEQ ID NO: 8 - DNA, 6146 bp, Artificial Sequence
  pAAV-tnt-GFP-CX43 vector sequence
ctgcgcgctcgctcgctcactgaggccgcccgggcaaagcccgggcgtcgggcgacctttggtcgcccggcctcagtgagcgagcgagcgcgcagagagggagtggccaactccatcactaggggttccttgtagttaatgattaacccgccatgctacttatctaccagggtaatggggatcctctagaactatagctagaattcgcccttacgggccccccctcgaggtcgggataaaagcagtctgggctttcacatgacagcatctggggctgcggcagagggtcgggtccgaagcgctgccttatcagcgtccccagccctgggaggtgacagctggctggcttgtgtcagcccctcgggcactcacgtatctccgtccgacgggtttaaaatagcaaaactctgaggccacacaatagcttgggcttatatgggctcctgtgggggaagggggagcacggagggggccggggccgctgctgccaaaatagcagctcacaagtgttgcattcctctctgggcgccgggcacattcctgctggctctgcccgccccggggtgggcgccggggggaccttaaagcctctgccccccaaggagcccttcccagacagccgccggcacccaccgctccgtgggacgatccccgaagctctagagctttattgcggtagtttatcacagttaaattgctaacgcagtcagtgcttctgacacaacagtggtcgtgaggcactgggcaggtaagtatcaaggttacaagacaggtttaaggagaccaatagaaactgggcttgtcgagacagagaagactcttgcgtttctgataggcacctattggtcttactgacatccactttgcctttctctccacaggtgtccactcccagttcaattacagctcttaaggctagagtacttaatacgactcactataggctagcgctaccggtcgccaccatggtgagcaagggcgccgagctgttcaccggcatcgtgcccatcctgatcgagctgaatggcgatgtgaatggccacaagttcagcgtgagcggcgagggcgagggcgatgccacctacggcaagctgaccctgaagttcatctgcaccaccggcaagctgcctgtgccctggcccaccctggtgaccaccctgagctacggcgtgcagtgcttctcacgctaccccgatcacatgaagcagcacgacttcttcaagagcgccatgcctgagggctacatccaggagcgcaccatcttcttcgaggatgacggcaactacaagtcgcgcgccgaggtgaagttcgagggcgataccctggtgaatcgcatcgagctgaccggcaccgatttcaaggaggatggcaacatcctgggcaataagatggagtacaactacaacgcccacaatgtgtacatcatgaccgacaaggccaagaatggcatcaaggtgaacttcaagatccgccacaacatcgaggatggcagcgtgcagctggccgaccactaccagcagaatacccccatcggcgatggccctgtgctgctgcccgataaccactacctgtccacccagagcgccctgtccaaggaccccaacgagaagcgcgatcacatgatctacttcggcttcgtgaccgccgccgccatcacccacggcatggatgagctgtacaagtccggactcagatctcgagctcaagcttcgaattctgcagtcgacggtaccgagctcggatccactagtaacggccgccagtgtgctggaattcggcttatgggtgactggagcgccttaggcaaactccttgacaaggttcaagcctactcaactgctggagggaaggtgtggctgtcagtacttttcattttccgaatcctgctgctggggacagcggttgagtcagcctggggagatgagcagtctgcctttcgttgtaacactcagcaacctggttgtgaaaatgtctgctatgacaagtctttcccaatctctcatgtgcgcttctgggtcctgcagatcatatttgtgtctgtacccacactcttgtacctggctcatgtgttctatgtgatgcgaaaggaagagaaactgaacaagaaagaggaagaactcaaggttgcccaaactgatggtgtcaatgtggacatgcacttgaagcagattgagataaagaagttcaagtacggtattgaagagcatggtaaggtgaaaatgcgaggggggttgctgcgaacctacatcatcagtatcctcttcaagtctatctttgaggtggccttcttgctgatccagtggtacatctatggattcagcttgagtgctgtttacacttgcaaaagagatccctgcccacatcaggtggactgtttcctctctcgccccacggagaaaaccatcttcatcatcttcatgctggtggtgtccttggtgtccctggccttgaatatcattgaactcttctatgttttcttcaagggcgttaaggatcgggttaagggaaagagcgacccttaccatgcgaccagtggtgcgctgagccctgccaaagactgtgggtctcaaaaatatgcttatttcaatggctgctcctcaccaaccgctcccctctcgcctatgtctcctcctgggtacaagctggttactggcgacagaaacaattcttcttgccgcaattacaacaagcaagcaagtgagcaaaactgggctaattacagtgcagaacaaaatcgaatggggcaggcgggaagcaccatctctaactcccatgcacagccttttgatttccccgatgataaccagaattcaaaaaaactagctgctggacatgaattacagccactagccattgtggaccagcgaccttcaagcagagccagcagtcgtgccagcagcagacctcggcctgatgacctggagatctaatctaggacccgggcggcctcgaggacggggtgaactacgcctgaggatccgatctttttccctctgccaaaaattatggggacatcatgaagccccttgagcatctgacttctggctaataaaggaaatttattttcattgcaatagtgtgttggaattttttgtgtctctcactcggaagcaattcgttgatctgaatttcgaccacccataatacccattaccctggtagataagtagcatggcgggttaatcattaactacaaggaacccctagtgatggagttggccactccctctctgcgcgctcgctcgctcactgaggccgggcgaccaaaggtcgcccgacgcccgggctttgcccgggcggcctcagtgagcgagcgagcgcgcagccttaattaacctaattcactggccgtcgttttacaacgtcgtgactgggaaaaccctggcgttacccaacttaatcgccttgcagcacatccccctttcgccagctggcgtaatagcgaagaggcccgcaccgatcgcccttcccaacagttgcgcagcctgaatggcgaatgggacgcgccctgtagcggcgcattaagcgcggcgggtgtggtggttacgcgcagcgtgaccgctacacttgccagcgccctagcgcccgctcctttcgctttcttcccttcctttctcgccacgttcgccggctttccccgtcaagctctaaatcgggggctccctttagggttccgatttagtgctttacggcacctcgaccccaaaaaacttgattagggtgatggttcacgtagtgggccatcgccctgatagacggtttttcgccctttgacgttggagtccacgttctttaatagtggactcttgttccaaactggaacaacactcaaccctatctcggtctattcttttgatttataagggattttgccgatttcggcctattggttaaaaaatgagctgatttaacaaaaatttaacgcgaattttaacaaaatattaacgcttacaatttaggtggcacttttcggggaaatgtgcgcggaacccctatttgtttatttttctaaatacattcaaatatgtatccgctcatgagacaataaccctgataaatgcttcaataatattgaaaaaggaagagtatgagtattcaacatttccgtgtcgcccttattcccttttttgcggcattttgccttcctgtttttgctcacccagaaacgctggtgaaagtaaaagatgctgaagatcagttgggtgcacgagtgggttacatcgaactggatctcaacagcggtaagatccttgagagttttcgccccgaagaacgttttccaatgatgagcacttttaaagttctgctatgtggcgcggtattatcccgtattgacgccgggcaagagcaactcggtcgccgcatacactattctcagaatgacttggttgagtactcaccagtcacagaaaagcatcttacggatggcatgacagtaagagaattatgcagtgctgccataaccatgagtgataacactgcggccaacttacttctgacaacgatcggaggaccgaaggagctaaccgcttttttgcacaacatgggggatcatgtaactcgccttgatcgttgggaaccggagctgaatgaagccataccaaacgacgagcgtgacaccacgatgcctgtagcaatggcaacaacgttgcgcaaactattaactggcgaactacttactctagcttcccggcaacaattaatagactggatggaggcggataaagttgcaggaccacttctgcgctcggcccttccggctggctggtttattgctgataaatctggagccggtgagcgtgggtctcgcggtatcattgcagcactggggccagatggtaagccctcccgtatcgtagttatctacacgacggggagtcaggcaactatggatgaacgaaatagacagatcgctgagataggtgcctcactgattaagcattggtaactgtcagaccaagtttactcatatatactttagattgatttaaaacttcatttttaatttaaaaggatctaggtgaagatcctttttgataatctcatgaccaaaatcccttaacgtgagttttcgttccactgagcgtcagaccccgtagaaaagatcaaaggatcttcttgagatcctttttttctgcgcgtaatctgctgcttgcaaacaaaaaaaccaccgctaccagcggtggtttgtttgccggatcaagagctaccaactctttttccgaaggtaactggcttcagcagagcgcagataccaaatactgttcttctagtgtagccgtagttaggccaccacttcaagaactctgtagcaccgcctacatacctcgctctgctaatcctgttaccagtggctgctgccagtggcgataagtcgtgtcttaccgggttggactcaagacgatagttaccggataaggcgcagcggtcgggctgaacggggggttcgtgcacacagcccagcttggagcgaacgacctacaccgaactgagatacctacagcgtgagctatgagaaagcgccacgcttcccgaagggagaaaggcggacaggtatccggtaagcggcagggtcggaacaggagagcgcacgagggagcttccagggggaaacgcctggtatctttatagtcctgtcgggtttcgccacctctgacttgagcgtcgatttttgtgatgctcgtcaggggggcggagcctatggaaaaacgccagcaacgcggcctttttacggttcctggccttttgctggccttttgctcacatgttctttcctgcgttatcccctgattctgtggataaccgtattaccgcctttgagtgagctgataccgctcgccgcagccgaacgaccgagcgcagcgagtcagtgagcgaggaagcggaagagcgcccaatacgcaaaccgcctctccccgcgcgttggccgattcattaatgcagctggcacgacaggtttcccgactggaaagcgggcagtgagcgcaacgcaattaatgtgagttagctcactcattaggcaccccaggctttacactttatgcttccggctcgtatgttgtgtggaattgtgagcggataacaatttcacacaggaaacagctatgaccatgattacgccagatttaattaaggccttaattagg

SEQ ID NO: 9 - DNA, 849 bp, Homo sapiens
atgcgaaaggaagagaaactgaacaagaaagaggaagaactcaaggttgcccaaactgatggtgtcaatgtggacatgcacttgaagcagattgagataaagaagttcaagtacggtattgaagagcatggtaaggtgaaaatgcgaggggggttgctgcgaacctacatcatcagtatcctcttcaagtctatctttgaggtggccttcttgctgatccagtggtacatctatggattcagcttgagtgctgtttacacttgcaaaagagatccctgcccacatcaggtggactgtttcctctctcgccccacggagaaaaccatcttcatcatcttcatgctggtggtgtccttggtgtccctggccttgaatatcattgaactcttctatgttttcttcaagggcgttaaggatcgggttaagggaaagagcgacccttaccatgcgaccagtggtgcgctgagccctgccaaagactgtgggtctcaaaaatatgcttatttcaatggctgctcctcaccaaccgctcccctctcgcctatgtctcctcctgggtacaagctggttactggcgacagaaacaattcttcttgccgcaattacaacaagcaagcaagtgagcaaaactgggctaattacagtgcagaacaaaatcgaatggggcaggcgggaagcaccatctctaactcccatgcacagccttttgatttccccgatgataaccagaattctaaaaaactagctgctggacatgaattacagccactagccattgtggaccagcgaccttcaagcagagccagcagtcgtgccagcagcagacctcggcctgatgacctggagatc

SEQ ID NO: 10 - DNA, 774 bp, Homo sapiens
atgcacttgaagcagattgagataaagaagttcaagtacggtattgaagagcatggtaaggtgaaaatgcgaggggggttgctgcgaacctacatcatcagtatcctcttcaagtctatctttgaggtggccttcttgctgatccagtggtacatctatggattcagcttgagtgctgtttacacttgcaaaagagatccctgcccacatcaggtggactgtttcctctctcgccccacggagaaaaccatcttcatcatcttcatgctggtggtgtccttggtgtccctggccttgaatatcattgaactcttctatgttttcttcaagggcgttaaggatcgggttaagggaaagagcgacccttaccatgcgaccagtggtgcgctgagccctgccaaagactgtgggtctcaaaaatatgcttatttcaatggctgctcctcaccaaccgctcccctctcgcctatgtctcctcctgggtacaagctggttactggcgacagaaacaattcttcttgccgcaattacaacaagcaagcaagtgagcaaaactgggctaattacagtgcagaacaaaatcgaatggggcaggcgggaagcaccatctctaactcccatgcacagccttttgatttccccgatgataaccagaattctaaaaaactagctgctggacatgaattacagccactagccattgtggaccagcgaccttcaagcagagccagcagtcgtgccagcagcagacctcggcctgatgacctggagatc

SEQ ID NO: 11 - DNA, 708 bp, Homo sapiens
atgcgaggggggttgctgcgaacctacatcatcagtatcctcttcaagtctatctttgaggtggccttcttgctgatccagtggtacatctatggattcagcttgagtgctgtttacacttgcaaaagagatccctgcccacatcaggtggactgtttcctctctcgccccacggagaaaaccatcttcatcatcttcatgctggtggtgtccttggtgtccctggccttgaatatcattgaactcttctatgttttcttcaagggcgttaaggatcgggttaagggaaagagcgacccttaccatgcgaccagtggtgcgctgagccctgccaaagactgtgggtctcaaaaatatgcttatttcaatggctgctcctcaccaaccgctcccctctcgcctatgtctcctcctgggtacaagctggttactggcgacagaaacaattcttcttgccgcaattacaacaagcaagcaagtgagcaaaactgggctaattacagtgcagaacaaaatcgaatggggcaggcgggaagcaccatctctaactcccatgcacagccttttgatttccccgatgataaccagaattctaaaaaactagctgctggacatgaattacagccactagccattgtggaccagcgaccttcaagcagagccagcagtcgtgccagcagcagacctcggcctgatgacctggagatc

SEQ ID NO: 12 - DNA, 510 bp, Homo sapiens
atgctggtggtgtccttggtgtccctggccttgaatatcattgaactcttctatgttttcttcaagggcgttaaggatcgggttaagggaaagagcgacccttaccatgcgaccagtggtgcgctgagccctgccaaagactgtgggtctcaaaaatatgcttatttcaatggctgctcctcaccaaccgctcccctctcgcctatgtctcctcctgggtacaagctggttactggcgacagaaacaattcttcttgccgcaattacaacaagcaagcaagtgagcaaaactgggctaattacagtgcagaacaaaatcgaatggggcaggcgggaagcaccatctctaactcccatgcacagccttttgatttccccgatgataaccagaattctaaaaaactagctgctggacatgaattacagccactagccattgtggaccagcgaccttcaagcagagccagcagtcgtgccagcagcagacctcggcctgatgacctggagatc